European Patent Application EP 4 286 406 A1, published December 6, 2023. Title: Fusion molecules that induce non-inflammatory phagocytosis. Applicant: KOREA ADVANCED INSTITUTE OF SCIENCE AND TECHNOLOGY. The sequence listing filed with the application follows.

SEQUENCE LISTING (6 sequences)

SEQ ID NO: 1 - protein, 173 aa, Artificial Sequence
  amino acid sequence
GRMFSGTPVIRLRFKRLQPTRLVAEFDFRTFDPEGILLFAGGHQDSTWIVLALRAGRLELQLRYNGVGRVTSSGPVINHGMWQTISVEELARNLVIKVNRDAVMKIAVAGDLFQPERGLYHLNLTVGGIPFHEKDLVQPINPRLDGCMRSWNWLNGEDTTIQETVKVNTRMQC

SEQ ID NO: 2 - protein, 194 aa, Artificial Sequence
  Gas6 derived LG2
GSFYPGSGFAFYSLDYMRTPLDVGTESTWEVEVVAHIRPAADTGVLFALWAPDLRAVPLSVALVDYHSTKKLKKQLVVLAVEHTALALMEIKVCDGQEHVVTVSLRDGEATLEVDGTRGQSEVSAAQLQERLAVLERHLRSPVLTFAGGLPDVPVTSAPVTAFYRGCMTLEVNRRLLDLDEAAYKHSDITAHSC

SEQ ID NO: 3 - protein, 177 aa, Artificial Sequence
  amino acid sequence
LLYLAEQFAGVVLYLKFRLPEISRFSAEFDFRTYDSEGVILYAESIDHSAWLLIALRGGKIEVQLKNEHTSKITTGGDVINNGLWNMVSVEELEHSISIKIAKEAVMDINKPGPLFKPENGLLETKVYFAGFPRKVESELIKPINPRLDGCIRSWNLMKQGASGIKEIIQEKQNKHC

SEQ ID NO: 4 - protein, 183 aa, Artificial Sequence
  amino acid sequence
YYPGSGIAQFHIDYNNVSSAEGWHVNVTLNIRPSTGTGVMLALVSGNNTVPFAVSLVDSTSEKSQDILLSVENTVIYRIQALSLCSDQQSHLEFRVNRNNLELSTPLKIETISHEDLQRQLAVLDKAMKAKVATYLGGLPDVPFSATPVNAFYNGCMEVNINGVQLDLDEAISKHNDIRAHSC

SEQ ID NO: 5 - protein, 400 aa, Artificial Sequence
  amino acid sequence
DILPCVPFSVAKSVKSLYLGRMFSGTPVIRLRFKRLQPTRLVAEFDFRTFDPEGILLFAGGHQDSTWIVLALRAGRLELQLRYNGVGRVTSSGPVINHGMWQTISVEELARNLVIKVNRDAVMKIAVAGDLFQPERGLYHLNLTVGGIPFHEKDLVQPINPRLDGCMRSWNWLNGEDTTIQETVKVNTRMQCFSVTERGSFYPGSGFAFYSLDYMRTPLDVGTESTWEVEVVAHIRPAADTGVLFALWAPDLRAVPLSVALVDYHSTKKLKKQLVVLAVEHTALALMEIKVCDGQEHVVTVSLRDGEATLEVDGTRGQSEVSAAQLQERLAVLERHLRSPVLTFAGGLPDVPVTSAPVTAFYRGCMTLEVNRRLLDLDEAAYKHSDITAHSCPPVEPAAA

SEQ ID NO: 6 - protein, 393 aa, Artificial Sequence
  amino acid sequence
VVSVCLPLNLDTKYELLYLAEQFAGVVLYLKFRLPEISRFSAEFDFRTYDSEGVILYAESIDHSAWLLIALRGGKIEVQLKNEHTSKITTGGDVINNGLWNMVSVEELEHSISIKIAKEAVMDINKPGPLFKPENGLLETKVYFAGFPRKVESELIKPINPRLDGCIRSWNLMKQGASGIKEIIQEKQNKHCLVTVEKGSYYPGSGIAQFHIDYNNVSSAEGWHVNVTLNIRPSTGTGVMLALVSGNNTVPFAVSLVDSTSEKSQDILLSVENTVIYRIQALSLCSDQQSHLEFRVNRNNLELSTPLKIETISHEDLQRQLAVLDKAMKAKVATYLGGLPDVPFSATPVNAFYNGCMEVNINGVQLDLDEAISKHNDIRAHSCPSVWKKTKNS